European Patent Application EP 4 506 460 A1, published February 12, 2025. Title: A Method for Transduction of Target Gene in Immune Cells. Applicant: GC cell. Application KR. The sequence listing filed with the application follows.

SEQUENCE LISTING (9 sequences)

SEQ ID NO: 1 - DNA, 20 bp, synthetic construct
  misc_feature 1..20: note = anti-HER2 scFv CAR F primer
  source 1..20: mol_type = other DNA
ggagttcaagggcagattcg

SEQ ID NO: 2 - DNA, 20 bp, synthetic construct
  misc_feature 1..20: note = anti-HER2 scFv CAR R primer
  source 1..20: mol_type = other DNA
cccagtagtccactctcacg

SEQ ID NO: 3 - DNA, 20 bp, synthetic construct
  misc_feature 1..20: note = anti-HER2 scFv CAR probe
  source 1..20: mol_type = other DNA
aaggccgaggacaccgccgt

SEQ ID NO: 4 - DNA, 23 bp, synthetic construct
  misc_feature 1..23: note = RPPH1 F primer
  source 1..23: mol_type = other DNA
ccctagtctcagaccttcccaag

SEQ ID NO: 5 - DNA, 19 bp, synthetic construct
  misc_feature 1..19: note = RPPH1 R primer
  source 1..19: mol_type = other DNA
gcggagggaagctcatcag

SEQ ID NO: 6 - DNA, 24 bp, synthetic construct
  misc_feature 1..24: note = RPPH1 probe
  source 1..24: mol_type = other DNA
ccacgagctgagtgcgtcctgtca

SEQ ID NO: 7 - DNA, 20 bp, synthetic construct
  misc_feature 1..20: note = anti-CD19 or CD5 scFv CAR F primer
  source 1..20: mol_type = other DNA
cgggtcccactcgcaaacac

SEQ ID NO: 8 - DNA, 20 bp, synthetic construct
  misc_feature 1..20: note = anti-CD19 or CD5 scFv CAR R primer
  source 1..20: mol_type = other DNA
cggcctacaggtcagagaga

SEQ ID NO: 9 - DNA, 20 bp, synthetic construct
  misc_feature 1..20: note = anti-CD19 or CD5 scFv CAR probe
  source 1..20: mol_type = other DNA
ggcagcgttgccgacattct